European Patent Application EP 4 134 086 A1, published February 15, 2023. Title: HUMAN MACROPHAGES RESISTENT TO TUMOR_INDUCED REPOLARIZATION. Applicant: Technische Universität Dresden CNRS Universite d'Aix-Marseille INSERM. The sequence listing filed with the application follows.

SEQUENCE LISTING (9 sequences)

SEQ ID NO: 1 - DNA, 99 bp, homo
  DNA encoding sgRNA for MAF-5'UTR
atctggcggagcggcggcgggttttagagctagaaatagcaagttaaaataaggctagtccgttatcaacttgaaaaagtggcaccgagtcggtgcttt

SEQ ID NO: 2 - DNA, 99 bp, homo
  DNA ecoding sgRNA for MAF-3'UTR
accctgataagtgctccgcggttttagagctagaaatagcaagttaaaataaggctagtccgttatcaacttgaaaaagtggcaccgagtcggtgcttt

SEQ ID NO: 3 - DNA, 99 bp, homo
  DNA encoding sgRNA for MAFB-5'UTR
cggccgcaaagtttcccggggttttagagctagaaatagcaagttaaaataaggctagtccgttatcaacttgaaaaagtggcaccgagtcggtgcttt

SEQ ID NO: 4 - DNA, 99 bp, homo
  DNA encoding sgRNA for MAFB-3'UTR
tgacctgtttgacttgagcggttttagagctagaaatagcaagttaaaataaggctagtccgttatcaacttgaaaaagtggcaccgagtcggtgcttt

SEQ ID NO: 5 - DNA, 99 bp, Artificial Sequence
  guide RNA part of SEQ ID Nr.1-4 (as DNA). n can be a, c, g or t and is replaced by the respective protospacer sequence
nnnnnnnnnnnnnnnnnnnngttttagagctagaaatagcaagttaaaataaggctagtccgttatcaacttgaaaaagtggcaccgagtcggtgcttt

SEQ ID NO: 6 - DNA, 20 bp, Homo sapiens
  The protospacer sequence of SEQ ID Nr.1
atctggcggagcggcggcgg

SEQ ID NO: 7 - DNA, 20 bp, Homo sapiens
  The protospacer sequence of SEQ ID Nr.2
accctgataagtgctccgcg

SEQ ID NO: 8 - DNA, 20 bp, Homo sapiens
  The protospacer sequence of SEQ ID Nr.3
cggccgcaaagtttcccggg

SEQ ID NO: 9 - DNA, 20 bp, Homo sapiens
  The protospacer sequence of SEQ ID Nr. 4
tgacctgtttgacttgagcg